European Patent Specification EP 4 507 708 B1, published October 15, 2025. Title: PEPTIDE UTILE POUR LE TRANSPORT DE MOLECULES AU TRAVERS DE BARRIERES CELLULAIRES. Applicant: UNIVERSITE GRENOBLE ALPES. The sequence listing filed with the application follows.

SEQUENCE LISTING (7 sequences)

SEQ ID NO: 1 - protein, 51 aa, synthetic construct
ARGGLNARGILETRPPHEGLNASNARGARGARGSERARGLYSILELYSLYS

SEQ ID NO: 2 - DNA, 51 bp, synthetic construct
  source 1..51: mol_type = other DNA
cgccagcgcatttggtttcagaaccgccgccgcagccgcaaaattaaaaaa

SEQ ID NO: 3 - protein, 363 aa, synthetic construct
GLNVALGLNLEUVALGLNSERGLYGLYGLYLEUVALGLNALAGLYGLYSERLEUARGLEUSERCYSALAALASERGLYARGTHRPHESERSERASPTHRLEUALATRPPHEARGGLNALAPROGLYLYSGLUARGGLUPHEVALALASERILESERPROSERGLYGLYVALTHRTYRTYRGLUASPSERVALLYSGLYARGPHETHRILESERARGASPASNSERLYSASNTHRVALLEULEUGLNMETASNSERLEUTHRPROGLUASPTHRALAVALTYRTYRCYSASNARGASPPROLYSTYRGLYASNTHRARGTYRTRPGLYGLNGLYTHRGLNVALTHRVALSERSERALAALAALA

SEQ ID NO: 4 - protein, 435 aa, synthetic construct
METGLNVALGLNLEUVALGLNSERGLYGLYGLYLEUVALGLNALAGLYGLYSERLEUARGLEUSERCYSALAALASERGLYARGTHRPHESERSERASPTHRLEUALATRPPHEARGGLNALAPROGLYLYSGLUARGGLUPHEVALALASERILESERPROSERGLYGLYVALTHRTYRTYRGLUASPSERVALLYSGLYARGPHETHRILESERARGASPASNSERLYSASNTHRVALLEULEUGLNMETASNSERLEUTHRPROGLUASPTHRALAVALTYRTYRCYSASNARGASPPROLYSTYRGLYASNTHRARGTYRTRPGLYGLNGLYTHRGLNVALTHRVALSERSERALAALAALAARGGLNARGILETRPPHEGLNASNARGARGARGSERARGLYSILELYSLYSHISHISHISHISHISHIS

SEQ ID NO: 5 - DNA, 438 bp, synthetic construct
  source 1..438: mol_type = other DNA
atgcaggtgcagctggtgcagtctgggggaggattggtgcaggctgggggttctctgagactctcctgtgcagcctctggacgcaccttcagtagcgataccctggcgtggttccgccaggcgccagggaaggagcgtgagtttgtagcgtctattagtcccagtggtggtgtcacatactatgaagactccgtgaagggccgattcaccatctccagagacaacagcaagaacacggtgttgctgcaaatgaacagcctgacacctgaggacacggccgtctattactgtaaccgggaccccaagtacggtaacactagatactggggccaggggacccaggtcaccgtctcctcagcggccgcacgccagcgcatttggtttcagaaccgccgccgcagccgcaaaattaaaaaacatcaccaccatcaccattaa

SEQ ID NO: 6 - protein, 6 aa, synthetic construct
RRPYIL

SEQ ID NO: 7 - protein, 23 aa, synthetic construct
RQRIWFQNRRRSRKIKKRRPYIL